European Patent Application EP 4 159 231 A1, published April 5, 2023. Title: Attenuating bacterial virulence by attenuating bacterial folate transport. Applicant: Smith, Hilde Ingebritson, Alaina Neubauer, Axel de Greeff, Astrid. The sequence listing filed with the application follows.

SEQUENCE LISTING (27 sequences)

SEQ ID NO: 1 - DNA, 30 bp, Artificial Sequence
  Primer comE1
cgagctcggaagaattggttattgcgcgtg

SEQ ID NO: 2 - DNA, 29 bp, Artificial Sequence
  Primer comE3
cgggatcccgggggatgacctgttgcttg

SEQ ID NO: 3 - DNA, 33 bp, Artificial Sequence
  Primer comE3
tcccccgggggagtcgtgtgtattcgacagcgg

SEQ ID NO: 4 - DNA, 31 bp, Artificial Sequence
  Primer comE4
tcccccgggggacaagcaacaggtcatcccc

SEQ ID NO: 5 - DNA, 29 bp, Artificial Sequence
  Primer comE6
cgggatcccggttgaatgcccggcaagcc

SEQ ID NO: 6 - DNA, 23 bp, Artificial Sequence
  Primer Orf2-fw
ctacggctggttcttctatcgaa

SEQ ID NO: 7 - DNA, 22 bp, Artificial Sequence
  Primer Orf2-rev
gcaatcggtgtcatgataaagg

SEQ ID NO: 8 - DNA, 20 bp, Artificial Sequence
  Primer folC-fw
gtttgtccgtccatcggttt

SEQ ID NO: 9 - DNA, 20 bp, Artificial Sequence
  Primer folC-rev
ctggtcggtcgcatagatga

SEQ ID NO: 10 - DNA, 21 bp, Artificial Sequence
  Primer RecA-fw
ggtttgcaggctcgtatgatg

SEQ ID NO: 11 - DNA, 23 bp, Artificial Sequence
  Primer RecA-rev
accaaacatgacaccgacttttt

SEQ ID NO: 12 - DNA, 51 bp, Artificial Sequence
  Primer t488a
gaaaggtatagtttttagcaagtggacaaaatatatagtgtgtgatacaat

SEQ ID NO: 13 - DNA, 51 bp, Artificial Sequence
  Primer t488a_antisense
attgtatcacacactatatattttgtccacttgctaaaaactatacctttc

SEQ ID NO: 14 - DNA, 24 bp, Artificial Sequence
  Primer V735-fw
tatgcgcaatgacgtagtagaagg

SEQ ID NO: 15 - DNA, 16 bp, Artificial Sequence
  Primer M13-rev
aacagctatgaccatg

SEQ ID NO: 16 - protein, 5 aa, Streptococcus suis
FYRKP

SEQ ID NO: 17 - protein, 168 aa, Clostridium bolteae
MTKTKHMVWMGILIAVSIVLSRFLSFSAWNVKIGFAFIPIVIGAVLFGPVQGGIAAAAADFLGAILFPIGMYFPGFTVTAFLTGLTYGILLHKNRSMFRIACAVLIVQLVYGLLLNTCWISLLYGAPYLALLSTRIVQYVVLIPVQFVIIARMYVLGSKKYHILQENS

SEQ ID NO: 18 - protein, 187 aa, Clostridium phytofermentans
MLNQEKNVKNKDLKKGKKVFTLETFIVLALLVAIEVILTRFLSLKEWNIRFSFGFIPVVIAAILYGPIASATVAACSDFLGAILFPMGAYFPGFTITAFISGIVYGLFLHKKQSLPNIVGAAVVNQFFCGLVINSYWLSIISGKSTFWGLIPIRSIQSAVMSIVIISVTYVISKTIVPIIKKAIVIM

SEQ ID NO: 19 - protein, 189 aa, Alkaliphilus metalliredigens
MKFNTRKLVTLSLLMALTIVFTRIASIRIPFGGVEGVRVGFGSLPILLAGILFGPISGFIVGALGDLIGYFLNPMGAYMPHFTLSAGLSGFIPGSIYYFTFRPKSNIHFSSKLQVSRPSFWLIFISILIGQVTISLLLIPYFLSALFSIPYELTIIPRTITQLISIPIFSWVIWIISNKTNIFDYVKSK

SEQ ID NO: 20 - protein, 162 aa, Thermoanaerobacter tengcongensis
MKKFTTREIAFLALLVALNIVLTRIASIRIAIGGVEGIRIGFGAFPVIFSGIAFGPYAGGIVGALGDIIGYFINPMGPYMPHFTFTAALVGILPPLFLKPFKAQIPTFWQLVIAIGLGQTISSIILTPYFIQMLFHLPMKITVPPRIVTQAIQVPLYAFLLK

SEQ ID NO: 21 - protein, 175 aa, Enterococcus faecium
HRLDARMIAIMGLLIALMVTLSRLVAIETPFIKISVTFIPQVIMGILFGPFWSGIGAVLADLVGMALFSKSAFFIGFTLNAFIEGAIYGFFFYRKEITWKNAILATLSVTLIINLFLTPLWLALMYHVPLFSWVVWAPRLLKTVIWLPIQSIAIYYVGRSIPYKKILRSLAIHAK

SEQ ID NO: 22 - protein, 179 aa, Enterococcus faecalis
MTKKKFGTKSIALMGVLIAVVVVFSRFFAYETTFLKISFTFIPESLIGMIFGPFWAGIGTAVADVVGMLLFPKAGYFPGFTLNAFLAGAIYGYFYYKKEMTWQRVILATLLVTVLINIILTPLWLSLMYGVNLANFAWWVPRLIKTVIFFPIQVIATYYLGNKIPFKRLFGKPLSELDQ

SEQ ID NO: 23 - protein, 177 aa, Lactobacillus brevis
MKTMAKTQLPKLDTLSMVTMGVLMALQLVISRFSVGNNFIKVSFTFLIVALIAKWFGPWWGMLTAAVVDVIGTLMTGGPFFIGFTVSAVLGSLIYAVFLYRQPVSWWRVIGASVLIALLVNTLLNTLWVTIMYQTPFWSLLPVRALKELIVTPVQIVLVYLLLKSQVIQMIQARLNK

SEQ ID NO: 24 - protein, 186 aa, Streptococcus mutans
MNTMFKSPKLSPQRLVTLAMLIALAFAIGKFSIPIIPQQLIISPTFIVNVMIGMIGGPIWAFISLAILDIVDNLSSGAGNFIIWWTLLEAVQGLFYGLFFYQKSLSWTNKKDWLHVTIATAIIMLIGSFIFTPLLVQIYYGVPFWAQFAAGRWLKIFEIPIRILVTMAIMPQLQRIPELRKLANFK

SEQ ID NO: 25 - protein, 186 aa, Streptococcus gallolyticus
MNLFFKTPKLTLKRLVSLAMLIALAFIVGKFSIPVIPQQLVVSLTFIVNTIIGMIGGPIWGFISLGILDVVDTLSSSSAGNFIIWWTLMEAIQGFFYGLFFYGKPLSWSSKKDWLHVTIATVVIMLIGTFILTPLLIQIYFGVPFWAQYLAGRWLKIFEIPLRIIITMLVIPRLQKIPELRKLANL

SEQ ID NO: 26 - protein, 185 aa, Streptococcus uberis
MPKQLYFPKLTVQRLVTLAMLIALAVIVSKFSVSIIPNQLVISFTFIVNTVIGIIAGPFWSFITLAMIDLIDSLMGGTSHFIIWWTVMEAFQGLLYGFFFYKRPLRSNQKKDWIYVSAVTLVIMLFSTFLITPLLIQIYFHVPFWAQYAAGRWFKIFEIPLRVLLTMFLIPPLQRIPEIKKLSAL

SEQ ID NO: 27 - protein, 183 aa, Streptococcus suis
MEKKIPKLTVQLLAAIAMTLALVMIVENYFSIRISDTLQVQFTFIPNTILGAIAGPVWAAVFAAISDPVFVLFSGQTVLFTWILIEAVSAFIYGWFFYRKPLDTKNKADWLYVAGVVVLIQVVISFIMTPIALHFHFGTPWIVLYSSRLIKAVFEIPLRIVVTMLVLPSLQKIPELAKLMGIK